European Patent Application EP 4 617 359 A1, published September 17, 2025. Title: 고당 반죽에서 발효력을 유지하는 사카로마이세스 세레비지에 FRUITFLY 균주. Applicant: 주식회사 르빵. Application KR. The sequence listing filed with the application follows.

SEQUENCE LISTING (1 sequence)

SEQ ID NO: 1 - DNA, 1433 bp, Saccharomyces cerevisiae
  source 1..1433: mol_type = genomic DNA
gtcctgcatgtctagtataagcatttatacagtgaaactgcgaatggctcattaaatcagttatcgtttatttgatagtaccttactacttggataaccgtggtaattctagagctaatacatgcttaaaatcccgactgtttggaagggatgtatttattagataaaaaatcaatgccttcgggctctttgatgattcataataacttttcgaatcgcatggccttgtgctggcgatggttcattcaaatttctgccctatcaactttcgatggtaggatagtggcctaccatggtttcaacgggtaacggggaataagggttcgattccggagagggagcctgagaaacggctaccacatccaaggaaggcagcaggcgcgcaaattacccaatcccgacacggggaggtagtgacaataaataacgatacagggcccttttgggtcttgtaattggaatgagtacaatgtaaataccttaacgaggaacaattggagggcaagtctggtgccagcagccgcggtaattccagctccaaaagcgtatattaaagttgttgcagttaaaaagctcgtagttgaaccttgggcttggctggccggtccatctttttgatgcgtactggacccagccgagcctttccttctgggtagccatttatggcgaaccaggacttttactttgaaaaaattagagtgttcaaagcaggcctttgctcgaatatattagcatggaataatagaataggacgttatggttctattttgttggtttctaggaccatcgtaatgattaatagggacggtcgggggtatcagtattcagttgtcagaggtgaaattcttggatttactgaagactaactactgcgaaagcattaaccaaggacgttttcattaatcaagaacgaaagttaggggatcgaagatgatcagatacccgtcgtagtcttaaccataactatgcgacaagggaaccggttgttgttcttttattgacgcaatcggcacttacagaatcaaatcttggtctgggggggggataatgttcgccagggtgaaacttaaggaattgtcggagggcccccccggaggggagcggcgggttatttgttcccccggggaaaccccccggccacccacaaggatgtgagaatgaagcttttgttttttgtggggggggggggggggggcgcccccccggggggggggggtgggtttgtgtgtgtaagagagaaaaacaaaaaccaaaaaagagggggggtgggggggtgttttttttaaaaaaaaaatattttctaaataaaaaaaaaaaaaaaaacccctctttttccccccccccccccccccccccatcccttggtgtttatattttttctggtgggggttttttttattatcaaaaaaaaaaaaaatttcttttccccccca